European Patent Specification EP 3 721 892 B1, published May 22, 2024. Title: METHODS AND COMPOSITIONS FOR TREATMENT OF DISORDERS WITH FOLLISTATIN POLYPEPTIDES. Applicant: ACCELERON PHARMA INC. Application PCT/US2015/034245. The sequence listing filed with the application follows.

SEQUENCE LISTING (47 sequences)

SEQ ID NO: 1 - protein, 317 aa, Homo sapiens
MVRARHQPGGLCLLLLLLCQFMEDRSAQAGNCWLRQAKNGRCQVLYKTELSKEECCSTGRLSTSWTEEDVNDNTLFKWMIFNGGAPNCIPCKETCENVDCGPGKKCRMNKKNKPRCVCAPDCSNITWKGPVCGLDGKTYRNECALLKARCKEQPELEVQYQGRCKKTCRDVFCPGSSTCVVDQTNNAYCVTCNRICPEPASSEQYLCGNDGVTYSSACHLRKATCLLGRSIGLAYEGKCIKAKSCEDIQCTGGKKCLWDFKVGRGRCSLCDELCPDSKSDEPVCASDNATYASECAMKEAACSSGVLLEVKHSGSCN

SEQ ID NO: 2 - protein, 288 aa, Homo sapiens
GNCWLRQAKNGRCQVLYKTELSKEECCSTGRLSTSWTEEDVNDNTLFKWMIFNGGAPNCIPCKETCENVDCGPGKKCRMNKKNKPRCVCAPDCSNITWKGPVCGLDGKTYRNECALLKARCKEQPELEVQYQGRCKKTCRDVFCPGSSTCVVDQTNNAYCVTCNRICPEPASSEQYLCGNDGVTYSSACHLRKATCLLGRSIGLAYEGKCIKAKSCEDIQCTGGKKCLWDFKVGRGRCSLCDELCPDSKSDEPVCASDNATYASECAMKEAACSSGVLLEVKHSGSCN

SEQ ID NO: 3 - protein, 344 aa, Homo sapiens
MVRARHQPGGLCLLLLLLCQFMEDRSAQAGNCWLRQAKNGRCQVLYKTELSKEECCSTGRLSTSWTEEDVNDNTLFKWMIFNGGAPNCIPCKETCENVDCGPGKKCRMNKKNKPRCVCAPDCSNITWKGPVCGLDGKTYRNECALLKARCKEQPELEVQYQGRCKKTCRDVFCPGSSTCVVDQTNNAYCVTCNRICPEPASSEQYLCGNDGVTYSSACHLRKATCLLGRSIGLAYEGKCIKAKSCEDIQCTGGKKCLWDFKVGRGRCSLCDELCPDSKSDEPVCASDNATYASECAMKEAACSSGVLLEVKHSGSCNSISEDTEEEEEDEDQDYSFPISSILEW

SEQ ID NO: 4 - protein, 315 aa, Homo sapiens
GNCWLRQAKNGRCQVLYKTELSKEECCSTGRLSTSWTEEDVNDNTLFKWMIFNGGAPNCIPCKETCENVDCGPGKKCRMNKKNKPRCVCAPDCSNITWKGPVCGLDGKTYRNECALLKARCKEQPELEVQYQGRCKKTCRDVFCPGSSTCVVDQTNNAYCVTCNRICPEPASSEQYLCGNDGVTYSSACHLRKATCLLGRSIGLAYEGKCIKAKSCEDIQCTGGKKCLWDFKVGRGRCSLCDELCPDSKSDEPVCASDNATYASECAMKEAACSSGVLLEVKHSGSCNSISEDTEEEEEDEDQDYSFPISSILEW

SEQ ID NO: 5 - protein, 12 aa, Homo sapiens
KKCRMNKKNKPR

SEQ ID NO: 6 - protein, 12 aa, Artificial Sequence
  Description of Artificial Sequence: Synthetic peptide
  MOD_RES (1)..(2): Any basic amino acid, particularly Lys or Arg
  MOD_RES (3)..(3): Any amino acid
  MOD_RES (4)..(4): Any basic amino acid, particularly Lys or Arg
  MOD_RES (5)..(6): Any amino acid
  MOD_RES (7)..(8): Any basic amino acid, particularly Lys or Arg
  MOD_RES (9)..(9): Any amino acid
  MOD_RES (10)..(10): Any basic amino acid, particularly Lys or Arg
  MOD_RES (11)..(11): Any amino acid
  MOD_RES (12)..(12): Any basic amino acid, particularly Lys or Arg
XXXXXXXXXXXX

SEQ ID NO: 7 - protein, 65 aa, Artificial Sequence
  Description of Artificial Sequence: Synthetic polypeptide
GNCWLRQAKNGRCQVLYKTELSKEECCSTGRLSTSWTEEDVNDNTLFKWMIFNGGAPNCIPCKET

SEQ ID NO: 8 - protein, 63 aa, Artificial Sequence
  Description of Artificial Sequence: Synthetic polypeptide
CWLRQAKNGRCQVLYKTELSKEECCSTGRLSTSWTEEDVNDNTLFKWMIFNGGAPNCIPCKET

SEQ ID NO: 9 - protein, 70 aa, Artificial Sequence
  Description of Artificial Sequence: Synthetic polypeptide
CENVDCGPGKKCRMNKKNKPRCVCAPDCSNITWKGPVCGLDGKTYRNECALLKARCKEQPELEVQYQGRC

SEQ ID NO: 10 - protein, 133 aa, Artificial Sequence
  Description of Artificial Sequence: Synthetic polypeptide
CWLRQAKNGRCQVLYKTELSKEECCSTGRLSTSWTEEDVNDNTLFKWMIFNGGAPNCIPCKETCENVDCGPGKKCRMNKKNKPRCVCAPDCSNITWKGPVCGLDGKTYRNECALLKARCKEQPELEVQYQGRC

SEQ ID NO: 11 - protein, 206 aa, Artificial Sequence
  Description of Artificial Sequence: Synthetic polypeptide
CWLRQAKNGRCQVLYKTELSKEECCSTGRLSTSWTEEDVNDNTLFKWMIFNGGAPNCIPCKETCENVDCGPGKKCRMNKKNKPRCVCAPDCSNITWKGPVCGLDGKTYRNECALLKARCKEQPELEVQYQGRCKKTCENVDCGPGKKCRMNKKNKPRCVCAPDCSNITWKGPVCGLDGKTYRNECALLKARCKEQPELEVQYQGRC

SEQ ID NO: 12 - protein, 145 aa, Artificial Sequence
  Description of Artificial Sequence: Synthetic polypeptide
CENVDCGPGKKCRMNKKNKPRCVCAPDCSNITWKGPVCGLDGKTYRNECALLKARCKEQPELEVQYQGRCKKTCRDVFCPGSSTCVVDQTNNAYCVTCNRICPEPASSEQYLCGNDGVTYSSACHLRKATCLLGRSIGLAYEGKC

SEQ ID NO: 13 - protein, 208 aa, Artificial Sequence
  Description of Artificial Sequence: Synthetic polypeptide
CWLRQAKNGRCQVLYKTELSKEECCSTGRLSTSWTEEDVNDNTLFKWMIFNGGAPNCIPCKETCENVDCGPGKKCRMNKKNKPRCVCAPDCSNITWKGPVCGLDGKTYRNECALLKARCKEQPELEVQYQGRCKKTCRDVFCPGSSTCVVDQTNNAYCVTCNRICPEPASSEQYLCGNDGVTYSSACHLRKATCLLGRSIGLAYEGKC

SEQ ID NO: 14 - protein, 320 aa, Homo sapiens
MVRARHQPGGLCLLLLLLCQFMEDRSAQAGNCWLRQAKNGRCQVLYKTELSKEECCSTGRLSTSWTEEDVNDNTLFKWMIFNGGAPNCIPCKETCENVDCGPGKKCRMNKKNKPRCVCAPDCSNITWKGPVCGLDGKTYRNECALLKARCKEQPELEVQYQGRCKKTCRDVFCPGSSTCVVDQTNNAYCVTCNRICPEPASSEQYLCGNDGVTYSSACHLRKATCLLGRSIGLAYEGKCIKAKSCEDIQCTGGKKCLWDFKVGRGRCSLCDELCPDSKSDEPVCASDNATYASECAMKEAACSSGVLLEVKHSGSCNSIS

SEQ ID NO: 15 - protein, 291 aa, Homo sapiens
GNCWLRQAKNGRCQVLYKTELSKEECCSTGRLSTSWTEEDVNDNTLFKWMIFNGGAPNCIPCKETCENVDCGPGKKCRMNKKNKPRCVCAPDCSNITWKGPVCGLDGKTYRNECALLKARCKEQPELEVQYQGRCKKTCRDVFCPGSSTCVVDQTNNAYCVTCNRICPEPASSEQYLCGNDGVTYSSACHLRKATCLLGRSIGLAYEGKCIKAKSCEDIQCTGGKKCLWDFKVGRGRCSLCDELCPDSKSDEPVCASDNATYASECAMKEAACSSGVLLEVKHSGSCNSIS

SEQ ID NO: 16 - protein, 289 aa, Homo sapiens
CWLRQAKNGRCQVLYKTELSKEECCSTGRLSTSWTEEDVNDNTLFKWMIFNGGAPNCIPCKETCENVDCGPGKKCRMNKKNKPRCVCAPDCSNITWKGPVCGLDGKTYRNECALLKARCKEQPELEVQYQGRCKKTCRDVFCPGSSTCVVDQTNNAYCVTCNRICPEPASSEQYLCGNDGVTYSSACHLRKATCLLGRSIGLAYEGKCIKAKSCEDIQCTGGKKCLWDFKVGRGRCSLCDELCPDSKSDEPVCASDNATYASECAMKEAACSSGVLLEVKHSGSCNSIS

SEQ ID NO: 17 - protein, 225 aa, Homo sapiens
THTCPPCPAPELLGGPSVFLFPPKPKDTLMISRTPEVTCVVVDVSHEDPEVKFNWYVDGVEVHNAKTKPREEQYNSTYRVVSVLTVLHQDWLNGKEYKCKVSNKALPAPIEKTISKAKGQPREPQVYTLPPSREEMTKNQVSLTCLVKGFYPSDIAVEWESNGQPENNYKTTPPVLDSDGSFFLYSKLTVDKSRWQQGNVFSCSVMHEALHNHYTQKSLSLSPGK

SEQ ID NO: 18 - protein, 223 aa, Homo sapiens
VECPPCPAPPVAGPSVFLFPPKPKDTLMISRTPEVTCVVVDVSHEDPEVQFNWYVDGVEVHNAKTKPREEQFNSTFRVVSVLTVVHQDWLNGKEYKCKVSNKGLPAPIEKTISKTKGQPREPQVYTLPPSREEMTKNQVSLTCLVKGFYPSDIAVEWESNGQPENNYKTTPPMLDSDGSFFLYSKLTVDKSRWQQGNVFSCSVMHEALHNHYTQKSLSLSPGK

SEQ ID NO: 19 - DNA, 1032 bp, Homo sapiens
atggtccgcgcgaggcaccagccgggtgggctttgcctcctgctgctgctgctctgccagttcatggaggaccgcagtgcccaggctgggaactgctggctccgtcaagcgaagaacggccgctgccaggtcctgtacaagaccgaactgagcaaggaggagtgctgcagcaccggccggctgagcacctcgtggaccgaggaggacgtgaatgacaacacactcttcaagtggatgattttcaacgggggcgcccccaactgcatcccctgtaaagaaacgtgtgagaacgtggactgtggacctgggaaaaaatgccgaatgaacaagaagaacaaaccccgctgcgtctgcgccccggattgttccaacatcacctggaagggtccagtctgcgggctggatgggaaaacctaccgcaatgaatgtgcactcctaaaggcaagatgtaaagagcagccagaactggaagtccagtaccaaggcagatgtaaaaagacttgtcgggatgttttctgtccaggcagctccacatgtgtggtggaccagaccaataatgcctactgtgtgacctgtaatcggatttgcccagagcctgcttcctctgagcaatatctctgtgggaatgatggagtcacctactccagtgcctgccacctgagaaaggctacctgcctgctgggcagatctattggattagcctatgagggaaagtgtatcaaagcaaagtcctgtgaagatatccagtgcactggtgggaaaaaatgtttatgggatttcaaggttgggagaggccggtgttccctctgtgatgagctgtgccctgacagtaagtcggatgagcctgtctgtgccagtgacaatgccacttatgccagcgagtgtgccatgaaggaagctgcctgctcctcaggtgtgctactggaagtaaagcactccggatcttgcaactccatttcggaagacaccgaggaagaggaggaagatgaagaccaggactacagctttcctatatcttctattctagagtgg

SEQ ID NO: 20 - DNA, 945 bp, Homo sapiens
gggaactgctggctccgtcaagcgaagaacggccgctgccaggtcctgtacaagaccgaactgagcaaggaggagtgctgcagcaccggccggctgagcacctcgtggaccgaggaggacgtgaatgacaacacactcttcaagtggatgattttcaacgggggcgcccccaactgcatcccctgtaaagaaacgtgtgagaacgtggactgtggacctgggaaaaaatgccgaatgaacaagaagaacaaaccccgctgcgtctgcgccccggattgttccaacatcacctggaagggtccagtctgcgggctggatgggaaaacctaccgcaatgaatgtgcactcctaaaggcaagatgtaaagagcagccagaactggaagtccagtaccaaggcagatgtaaaaagacttgtcgggatgttttctgtccaggcagctccacatgtgtggtggaccagaccaataatgcctactgtgtgacctgtaatcggatttgcccagagcctgcttcctctgagcaatatctctgtgggaatgatggagtcacctactccagtgcctgccacctgagaaaggctacctgcctgctgggcagatctattggattagcctatgagggaaagtgtatcaaagcaaagtcctgtgaagatatccagtgcactggtgggaaaaaatgtttatgggatttcaaggttgggagaggccggtgttccctctgtgatgagctgtgccctgacagtaagtcggatgagcctgtctgtgccagtgacaatgccacttatgccagcgagtgtgccatgaaggaagctgcctgctcctcaggtgtgctactggaagtaaagcactccggatcttgcaactccatttcggaagacaccgaggaagaggaggaagatgaagaccaggactacagctttcctatatcttctattctagagtgg

SEQ ID NO: 21 - DNA, 864 bp, Homo sapiens
gggaactgctggctccgtcaagcgaagaacggccgctgccaggtcctgtacaagaccgaactgagcaaggaggagtgctgcagcaccggccggctgagcacctcgtggaccgaggaggacgtgaatgacaacacactcttcaagtggatgattttcaacgggggcgcccccaactgcatcccctgtaaagaaacgtgtgagaacgtggactgtggacctgggaaaaaatgccgaatgaacaagaagaacaaaccccgctgcgtctgcgccccggattgttccaacatcacctggaagggtccagtctgcgggctggatgggaaaacctaccgcaatgaatgtgcactcctaaaggcaagatgtaaagagcagccagaactggaagtccagtaccaaggcagatgtaaaaagacttgtcgggatgttttctgtccaggcagctccacatgtgtggtggaccagaccaataatgcctactgtgtgacctgtaatcggatttgcccagagcctgcttcctctgagcaatatctctgtgggaatgatggagtcacctactccagtgcctgccacctgagaaaggctacctgcctgctgggcagatctattggattagcctatgagggaaagtgtatcaaagcaaagtcctgtgaagatatccagtgcactggtgggaaaaaatgtttatgggatttcaaggttgggagaggccggtgttccctctgtgatgagctgtgccctgacagtaagtcggatgagcctgtctgtgccagtgacaatgccacttatgccagcgagtgtgccatgaaggaagctgcctgctcctcaggtgtgctactggaagtaaagcactccggatcttgcaac

SEQ ID NO: 22 - DNA, 876 bp, Homo sapiens
gggaactgctggctccgtcaagcgaagaacggccgctgccaggtcctgtacaagaccgaactgagcaaggaggagtgctgcagcaccggccggctgagcacctcgtggaccgaggaggacgtgaatgacaacacactcttcaagtggatgattttcaacgggggcgcccccaactgcatcccctgtaaagaaacgtgtgagaacgtggactgtggacctgggaaaaaatgccgaatgaacaagaagaacaaaccccgctgcgtctgcgccccggattgttccaacatcacctggaagggtccagtctgcgggctggatgggaaaacctaccgcaatgaatgtgcactcctaaaggcaagatgtaaagagcagccagaactggaagtccagtaccaaggcagatgtaaaaagacttgtcgggatgttttctgtccaggcagctccacatgtgtggtggaccagaccaataatgcctactgtgtgacctgtaatcggatttgcccagagcctgcttcctctgagcaatatctctgtgggaatgatggagtcacctactccagtgcctgccacctgagaaaggctacctgcctgctgggcagatctattggattagcctatgagggaaagtgtatcaaagcaaagtcctgtgaagatatccagtgcactggtgggaaaaaatgtttatgggatttcaaggttgggagaggccggtgttccctctgtgatgagctgtgccctgacagtaagtcggatgagcctgtctgtgccagtgacaatgccacttatgccagcgagtgtgccatgaaggaagctgcctgctcctcaggtgtgctactggaagtaaagcactccggatcttgcaactccatttcgtgg

SEQ ID NO: 23 - protein, 29 aa, Unknown
  Description of Unknown: Follistatin leader sequence
MVRARHQPGGLCLLLLLLCQFMEDRSAQA

SEQ ID NO: 24 - protein, 22 aa, Unknown
  Description of Unknown: Tissue plasminogen activator (TPA) sequence
MDAMKRGLCCVLLLCGAVFVSP

SEQ ID NO: 25 - protein, 21 aa, Apis mellifera
MKFLVNVALVFMVVYISYIYA

SEQ ID NO: 26 - protein, 546 aa, Artificial Sequence
  Description of Artificial Sequence: Synthetic polypeptide
MVRARHQPGGLCLLLLLLCQFMEDRSAQAGNCWLRQAKNGRCQVLYKTELSKEECCSTGRLSTSWTEEDVNDNTLFKWMIFNGGAPNCIPCKETCENVDCGPGKKCRMNKKNKPRCVCAPDCSNITWKGPVCGLDGKTYRNECALLKARCKEQPELEVQYQGRCKKTCRDVFCPGSSTCVVDQTNNAYCVTCNRICPEPASSEQYLCGNDGVTYSSACHLRKATCLLGRSIGLAYEGKCIKAKSCEDIQCTGGKKCLWDFKVGRGRCSLCDELCPDSKSDEPVCASDNATYASECAMKEAACSSGVLLEVKHSGSCNTGGGTHTCPPCPAPELLGGPSVFLFPPKPKDTLMISRTPEVTCVVVDVSHEDPEVKFNWYVDGVEVHNAKTKPREEQYNSTYRVVSVLTVLHQDWLNGKEYKCKVSNKALPAPIEKTISKAKGQPREPQVYTLPPSREEMTKNQVSLTCLVKGFYPSDIAVEWESNGQPENNYKTTPPVLDSDGSFFLYSKLTVDKSRWQQGNVFSCSVMHEALHNHYTQKSLSLSPGK

SEQ ID NO: 27 - protein, 517 aa, Artificial Sequence
  Description of Artificial Sequence: Synthetic polypeptide
GNCWLRQAKNGRCQVLYKTELSKEECCSTGRLSTSWTEEDVNDNTLFKWMIFNGGAPNCIPCKETCENVDCGPGKKCRMNKKNKPRCVCAPDCSNITWKGPVCGLDGKTYRNECALLKARCKEQPELEVQYQGRCKKTCRDVFCPGSSTCVVDQTNNAYCVTCNRICPEPASSEQYLCGNDGVTYSSACHLRKATCLLGRSIGLAYEGKCIKAKSCEDIQCTGGKKCLWDFKVGRGRCSLCDELCPDSKSDEPVCASDNATYASECAMKEAACSSGVLLEVKHSGSCNTGGGTHTCPPCPAPELLGGPSVFLFPPKPKDTLMISRTPEVTCVVVDVSHEDPEVKFNWYVDGVEVHNAKTKPREEQYNSTYRVVSVLTVLHQDWLNGKEYKCKVSNKALPAPIEKTISKAKGQPREPQVYTLPPSREEMTKNQVSLTCLVKGFYPSDIAVEWESNGQPENNYKTTPPVLDSDGSFFLYSKLTVDKSRWQQGNVFSCSVMHEALHNHYTQKSLSLSPGK

SEQ ID NO: 28 - protein, 515 aa, Artificial Sequence
  Description of Artificial Sequence: Synthetic polypeptide
CWLRQAKNGRCQVLYKTELSKEECCSTGRLSTSWTEEDVNDNTLFKWMIFNGGAPNCIPCKETCENVDCGPGKKCRMNKKNKPRCVCAPDCSNITWKGPVCGLDGKTYRNECALLKARCKEQPELEVQYQGRCKKTCRDVFCPGSSTCVVDQTNNAYCVTCNRICPEPASSEQYLCGNDGVTYSSACHLRKATCLLGRSIGLAYEGKCIKAKSCEDIQCTGGKKCLWDFKVGRGRCSLCDELCPDSKSDEPVCASDNATYASECAMKEAACSSGVLLEVKHSGSCNTGGGTHTCPPCPAPELLGGPSVFLFPPKPKDTLMISRTPEVTCVVVDVSHEDPEVKFNWYVDGVEVHNAKTKPREEQYNSTYRVVSVLTVLHQDWLNGKEYKCKVSNKALPAPIEKTISKAKGQPREPQVYTLPPSREEMTKNQVSLTCLVKGFYPSDIAVEWESNGQPENNYKTTPPVLDSDGSFFLYSKLTVDKSRWQQGNVFSCSVMHEALHNHYTQKSLSLSPGK

SEQ ID NO: 29 - protein, 573 aa, Artificial Sequence
  Description of Artificial Sequence: Synthetic polypeptide
MVRARHQPGGLCLLLLLLCQFMEDRSAQAGNCWLRQAKNGRCQVLYKTELSKEECCSTGRLSTSWTEEDVNDNTLFKWMIFNGGAPNCIPCKETCENVDCGPGKKCRMNKKNKPRCVCAPDCSNITWKGPVCGLDGKTYRNECALLKARCKEQPELEVQYQGRCKKTCRDVFCPGSSTCVVDQTNNAYCVTCNRICPEPASSEQYLCGNDGVTYSSACHLRKATCLLGRSIGLAYEGKCIKAKSCEDIQCTGGKKCLWDFKVGRGRCSLCDELCPDSKSDEPVCASDNATYASECAMKEAACSSGVLLEVKHSGSCNSISEDTEEEEEDEDQDYSFPISSILEWTGGGTHTCPPCPAPELLGGPSVFLFPPKPKDTLMISRTPEVTCVVVDVSHEDPEVKFNWYVDGVEVHNAKTKPREEQYNSTYRVVSVLTVLHQDWLNGKEYKCKVSNKALPAPIEKTISKAKGQPREPQVYTLPPSREEMTKNQVSLTCLVKGFYPSDIAVEWESNGQPENNYKTTPPVLDSDGSFFLYSKLTVDKSRWQQGNVFSCSVMHEALHNHYTQKSLSLSPGK

SEQ ID NO: 30 - protein, 544 aa, Artificial Sequence
  Description of Artificial Sequence: Synthetic polypeptide
GNCWLRQAKNGRCQVLYKTELSKEECCSTGRLSTSWTEEDVNDNTLFKWMIFNGGAPNCIPCKETCENVDCGPGKKCRMNKKNKPRCVCAPDCSNITWKGPVCGLDGKTYRNECALLKARCKEQPELEVQYQGRCKKTCRDVFCPGSSTCVVDQTNNAYCVTCNRICPEPASSEQYLCGNDGVTYSSACHLRKATCLLGRSIGLAYEGKCIKAKSCEDIQCTGGKKCLWDFKVGRGRCSLCDELCPDSKSDEPVCASDNATYASECAMKEAACSSGVLLEVKHSGSCNSISEDTEEEEEDEDQDYSFPISSILEWTGGGTHTCPPCPAPELLGGPSVFLFPPKPKDTLMISRTPEVTCVVVDVSHEDPEVKFNWYVDGVEVHNAKTKPREEQYNSTYRVVSVLTVLHQDWLNGKEYKCKVSNKALPAPIEKTISKAKGQPREPQVYTLPPSREEMTKNQVSLTCLVKGFYPSDIAVEWESNGQPENNYKTTPPVLDSDGSFFLYSKLTVDKSRWQQGNVFSCSVMHEALHNHYTQKSLSLSPGK

SEQ ID NO: 31 - protein, 542 aa, Artificial Sequence
  Description of Artificial Sequence: Synthetic polypeptide
CWLRQAKNGRCQVLYKTELSKEECCSTGRLSTSWTEEDVNDNTLFKWMIFNGGAPNCIPCKETCENVDCGPGKKCRMNKKNKPRCVCAPDCSNITWKGPVCGLDGKTYRNECALLKARCKEQPELEVQYQGRCKKTCRDVFCPGSSTCVVDQTNNAYCVTCNRICPEPASSEQYLCGNDGVTYSSACHLRKATCLLGRSIGLAYEGKCIKAKSCEDIQCTGGKKCLWDFKVGRGRCSLCDELCPDSKSDEPVCASDNATYASECAMKEAACSSGVLLEVKHSGSCNSISEDTEEEEEDEDQDYSFPISSILEWTGGGTHTCPPCPAPELLGGPSVFLFPPKPKDTLMISRTPEVTCVVVDVSHEDPEVKFNWYVDGVEVHNAKTKPREEQYNSTYRVVSVLTVLHQDWLNGKEYKCKVSNKALPAPIEKTISKAKGQPREPQVYTLPPSREEMTKNQVSLTCLVKGFYPSDIAVEWESNGQPENNYKTTPPVLDSDGSFFLYSKLTVDKSRWQQGNVFSCSVMHEALHNHYTQKSLSLSPGK

SEQ ID NO: 32 - protein, 544 aa, Artificial Sequence
  Description of Artificial Sequence: Synthetic polypeptide
MVRARHQPGGLCLLLLLLCQFMEDRSAQAGNCWLRQAKNGRCQVLYKTELSKEECCSTGRLSTSWTEEDVNDNTLFKWMIFNGGAPNCIPCKETCENVDCGPGKKCRMNKKNKPRCVCAPDCSNITWKGPVCGLDGKTYRNECALLKARCKEQPELEVQYQGRCKKTCRDVFCPGSSTCVVDQTNNAYCVTCNRICPEPASSEQYLCGNDGVTYSSACHLRKATCLLGRSIGLAYEGKCIKAKSCEDIQCTGGKKCLWDFKVGRGRCSLCDELCPDSKSDEPVCASDNATYASECAMKEAACSSGVLLEVKHSGSCNTGGGVECPPCPAPPVAGPSVFLFPPKPKDTLMISRTPEVTCVVVDVSHEDPEVQFNWYVDGVEVHNAKTKPREEQFNSTFRVVSVLTVVHQDWLNGKEYKCKVSNKGLPAPIEKTISKTKGQPREPQVYTLPPSREEMTKNQVSLTCLVKGFYPSDIAVEWESNGQPENNYKTTPPMLDSDGSFFLYSKLTVDKSRWQQGNVFSCSVMHEALHNHYTQKSLSLSPGK

SEQ ID NO: 33 - protein, 515 aa, Artificial Sequence
  Description of Artificial Sequence: Synthetic polypeptide
GNCWLRQAKNGRCQVLYKTELSKEECCSTGRLSTSWTEEDVNDNTLFKWMIFNGGAPNCIPCKETCENVDCGPGKKCRMNKKNKPRCVCAPDCSNITWKGPVCGLDGKTYRNECALLKARCKEQPELEVQYQGRCKKTCRDVFCPGSSTCVVDQTNNAYCVTCNRICPEPASSEQYLCGNDGVTYSSACHLRKATCLLGRSIGLAYEGKCIKAKSCEDIQCTGGKKCLWDFKVGRGRCSLCDELCPDSKSDEPVCASDNATYASECAMKEAACSSGVLLEVKHSGSCNTGGGVECPPCPAPPVAGPSVFLFPPKPKDTLMISRTPEVTCVVVDVSHEDPEVQFNWYVDGVEVHNAKTKPREEQFNSTFRVVSVLTVVHQDWLNGKEYKCKVSNKGLPAPIEKTISKTKGQPREPQVYTLPPSREEMTKNQVSLTCLVKGFYPSDIAVEWESNGQPENNYKTTPPMLDSDGSFFLYSKLTVDKSRWQQGNVFSCSVMHEALHNHYTQKSLSLSPGK

SEQ ID NO: 34 - protein, 513 aa, Artificial Sequence
  Description of Artificial Sequence: Synthetic polypeptide
CWLRQAKNGRCQVLYKTELSKEECCSTGRLSTSWTEEDVNDNTLFKWMIFNGGAPNCIPCKETCENVDCGPGKKCRMNKKNKPRCVCAPDCSNITWKGPVCGLDGKTYRNECALLKARCKEQPELEVQYQGRCKKTCRDVFCPGSSTCVVDQTNNAYCVTCNRICPEPASSEQYLCGNDGVTYSSACHLRKATCLLGRSIGLAYEGKCIKAKSCEDIQCTGGKKCLWDFKVGRGRCSLCDELCPDSKSDEPVCASDNATYASECAMKEAACSSGVLLEVKHSGSCNTGGGVECPPCPAPPVAGPSVFLFPPKPKDTLMISRTPEVTCVVVDVSHEDPEVQFNWYVDGVEVHNAKTKPREEQFNSTFRVVSVLTVVHQDWLNGKEYKCKVSNKGLPAPIEKTISKTKGQPREPQVYTLPPSREEMTKNQVSLTCLVKGFYPSDIAVEWESNGQPENNYKTTPPMLDSDGSFFLYSKLTVDKSRWQQGNVFSCSVMHEALHNHYTQKSLSLSPGK

SEQ ID NO: 35 - protein, 571 aa, Artificial Sequence
  Description of Artificial Sequence: Synthetic polypeptide
MVRARHQPGGLCLLLLLLCQFMEDRSAQAGNCWLRQAKNGRCQVLYKTELSKEECCSTGRLSTSWTEEDVNDNTLFKWMIFNGGAPNCIPCKETCENVDCGPGKKCRMNKKNKPRCVCAPDCSNITWKGPVCGLDGKTYRNECALLKARCKEQPELEVQYQGRCKKTCRDVFCPGSSTCVVDQTNNAYCVTCNRICPEPASSEQYLCGNDGVTYSSACHLRKATCLLGRSIGLAYEGKCIKAKSCEDIQCTGGKKCLWDFKVGRGRCSLCDELCPDSKSDEPVCASDNATYASECAMKEAACSSGVLLEVKHSGSCNSISEDTEEEEEDEDQDYSFPISSILEWTGGGVECPPCPAPPVAGPSVFLFPPKPKDTLMISRTPEVTCVVVDVSHEDPEVQFNWYVDGVEVHNAKTKPREEQFNSTFRVVSVLTVVHQDWLNGKEYKCKVSNKGLPAPIEKTISKTKGQPREPQVYTLPPSREEMTKNQVSLTCLVKGFYPSDIAVEWESNGQPENNYKTTPPMLDSDGSFFLYSKLTVDKSRWQQGNVFSCSVMHEALHNHYTQKSLSLSPGK

SEQ ID NO: 36 - protein, 542 aa, Artificial Sequence
  Description of Artificial Sequence: Synthetic polypeptide
GNCWLRQAKNGRCQVLYKTELSKEECCSTGRLSTSWTEEDVNDNTLFKWMIFNGGAPNCIPCKETCENVDCGPGKKCRMNKKNKPRCVCAPDCSNITWKGPVCGLDGKTYRNECALLKARCKEQPELEVQYQGRCKKTCRDVFCPGSSTCVVDQTNNAYCVTCNRICPEPASSEQYLCGNDGVTYSSACHLRKATCLLGRSIGLAYEGKCIKAKSCEDIQCTGGKKCLWDFKVGRGRCSLCDELCPDSKSDEPVCASDNATYASECAMKEAACSSGVLLEVKHSGSCNSISEDTEEEEEDEDQDYSFPISSILEWTGGGVECPPCPAPPVAGPSVFLFPPKPKDTLMISRTPEVTCVVVDVSHEDPEVQFNWYVDGVEVHNAKTKPREEQFNSTFRVVSVLTVVHQDWLNGKEYKCKVSNKGLPAPIEKTISKTKGQPREPQVYTLPPSREEMTKNQVSLTCLVKGFYPSDIAVEWESNGQPENNYKTTPPMLDSDGSFFLYSKLTVDKSRWQQGNVFSCSVMHEALHNHYTQKSLSLSPGK

SEQ ID NO: 37 - protein, 540 aa, Artificial Sequence
  Description of Artificial Sequence: Synthetic polypeptide
CWLRQAKNGRCQVLYKTELSKEECCSTGRLSTSWTEEDVNDNTLFKWMIFNGGAPNCIPCKETCENVDCGPGKKCRMNKKNKPRCVCAPDCSNITWKGPVCGLDGKTYRNECALLKARCKEQPELEVQYQGRCKKTCRDVFCPGSSTCVVDQTNNAYCVTCNRICPEPASSEQYLCGNDGVTYSSACHLRKATCLLGRSIGLAYEGKCIKAKSCEDIQCTGGKKCLWDFKVGRGRCSLCDELCPDSKSDEPVCASDNATYASECAMKEAACSSGVLLEVKHSGSCNSISEDTEEEEEDEDQDYSFPISSILEWTGGGVECPPCPAPPVAGPSVFLFPPKPKDTLMISRTPEVTCVVVDVSHEDPEVQFNWYVDGVEVHNAKTKPREEQFNSTFRVVSVLTVVHQDWLNGKEYKCKVSNKGLPAPIEKTISKTKGQPREPQVYTLPPSREEMTKNQVSLTCLVKGFYPSDIAVEWESNGQPENNYKTTPPMLDSDGSFFLYSKLTVDKSRWQQGNVFSCSVMHEALHNHYTQKSLSLSPGK

SEQ ID NO: 38 - protein, 549 aa, Artificial Sequence
  Description of Artificial Sequence: Synthetic polypeptide
MVRARHQPGGLCLLLLLLCQFMEDRSAQAGNCWLRQAKNGRCQVLYKTELSKEECCSTGRLSTSWTEEDVNDNTLFKWMIFNGGAPNCIPCKETCENVDCGPGKKCRMNKKNKPRCVCAPDCSNITWKGPVCGLDGKTYRNECALLKARCKEQPELEVQYQGRCKKTCRDVFCPGSSTCVVDQTNNAYCVTCNRICPEPASSEQYLCGNDGVTYSSACHLRKATCLLGRSIGLAYEGKCIKAKSCEDIQCTGGKKCLWDFKVGRGRCSLCDELCPDSKSDEPVCASDNATYASECAMKEAACSSGVLLEVKHSGSCNSISTGGGTHTCPPCPAPELLGGPSVFLFPPKPKDTLMISRTPEVTCVVVDVSHEDPEVKFNWYVDGVEVHNAKTKPREEQYNSTYRVVSVLTVLHQDWLNGKEYKCKVSNKALPAPIEKTISKAKGQPREPQVYTLPPSREEMTKNQVSLTCLVKGFYPSDIAVEWESNGQPENNYKTTPPVLDSDGSFFLYSKLTVDKSRWQQGNVFSCSVMHEALHNHYTQKSLSLSPGK

SEQ ID NO: 39 - protein, 520 aa, Artificial Sequence
  Description of Artificial Sequence: Synthetic polypeptide
GNCWLRQAKNGRCQVLYKTELSKEECCSTGRLSTSWTEEDVNDNTLFKWMIFNGGAPNCIPCKETCENVDCGPGKKCRMNKKNKPRCVCAPDCSNITWKGPVCGLDGKTYRNECALLKARCKEQPELEVQYQGRCKKTCRDVFCPGSSTCVVDQTNNAYCVTCNRICPEPASSEQYLCGNDGVTYSSACHLRKATCLLGRSIGLAYEGKCIKAKSCEDIQCTGGKKCLWDFKVGRGRCSLCDELCPDSKSDEPVCASDNATYASECAMKEAACSSGVLLEVKHSGSCNSISTGGGTHTCPPCPAPELLGGPSVFLFPPKPKDTLMISRTPEVTCVVVDVSHEDPEVKFNWYVDGVEVHNAKTKPREEQYNSTYRVVSVLTVLHQDWLNGKEYKCKVSNKALPAPIEKTISKAKGQPREPQVYTLPPSREEMTKNQVSLTCLVKGFYPSDIAVEWESNGQPENNYKTTPPVLDSDGSFFLYSKLTVDKSRWQQGNVFSCSVMHEALHNHYTQKSLSLSPGK

SEQ ID NO: 40 - protein, 518 aa, Artificial Sequence
  Description of Artificial Sequence: Synthetic polypeptide
CWLRQAKNGRCQVLYKTELSKEECCSTGRLSTSWTEEDVNDNTLFKWMIFNGGAPNCIPCKETCENVDCGPGKKCRMNKKNKPRCVCAPDCSNITWKGPVCGLDGKTYRNECALLKARCKEQPELEVQYQGRCKKTCRDVFCPGSSTCVVDQTNNAYCVTCNRICPEPASSEQYLCGNDGVTYSSACHLRKATCLLGRSIGLAYEGKCIKAKSCEDIQCTGGKKCLWDFKVGRGRCSLCDELCPDSKSDEPVCASDNATYASECAMKEAACSSGVLLEVKHSGSCNSISTGGGTHTCPPCPAPELLGGPSVFLFPPKPKDTLMISRTPEVTCVVVDVSHEDPEVKFNWYVDGVEVHNAKTKPREEQYNSTYRVVSVLTVLHQDWLNGKEYKCKVSNKALPAPIEKTISKAKGQPREPQVYTLPPSREEMTKNQVSLTCLVKGFYPSDIAVEWESNGQPENNYKTTPPVLDSDGSFFLYSKLTVDKSRWQQGNVFSCSVMHEALHNHYTQKSLSLSPGK

SEQ ID NO: 41 - protein, 547 aa, Artificial Sequence
  Description of Artificial Sequence: Synthetic polypeptide
MVRARHQPGGLCLLLLLLCQFMEDRSAQAGNCWLRQAKNGRCQVLYKTELSKEECCSTGRLSTSWTEEDVNDNTLFKWMIFNGGAPNCIPCKETCENVDCGPGKKCRMNKKNKPRCVCAPDCSNITWKGPVCGLDGKTYRNECALLKARCKEQPELEVQYQGRCKKTCRDVFCPGSSTCVVDQTNNAYCVTCNRICPEPASSEQYLCGNDGVTYSSACHLRKATCLLGRSIGLAYEGKCIKAKSCEDIQCTGGKKCLWDFKVGRGRCSLCDELCPDSKSDEPVCASDNATYASECAMKEAACSSGVLLEVKHSGSCNSISTGGGVECPPCPAPPVAGPSVFLFPPKPKDTLMISRTPEVTCVVVDVSHEDPEVQFNWYVDGVEVHNAKTKPREEQFNSTFRVVSVLTVVHQDWLNGKEYKCKVSNKGLPAPIEKTISKTKGQPREPQVYTLPPSREEMTKNQVSLTCLVKGFYPSDIAVEWESNGQPENNYKTTPPMLDSDGSFFLYSKLTVDKSRWQQGNVFSCSVMHEALHNHYTQKSLSLSPGK

SEQ ID NO: 42 - protein, 518 aa, Artificial Sequence
  Description of Artificial Sequence: Synthetic polypeptide
GNCWLRQAKNGRCQVLYKTELSKEECCSTGRLSTSWTEEDVNDNTLFKWMIFNGGAPNCIPCKETCENVDCGPGKKCRMNKKNKPRCVCAPDCSNITWKGPVCGLDGKTYRNECALLKARCKEQPELEVQYQGRCKKTCRDVFCPGSSTCVVDQTNNAYCVTCNRICPEPASSEQYLCGNDGVTYSSACHLRKATCLLGRSIGLAYEGKCIKAKSCEDIQCTGGKKCLWDFKVGRGRCSLCDELCPDSKSDEPVCASDNATYASECAMKEAACSSGVLLEVKHSGSCNSISTGGGVECPPCPAPPVAGPSVFLFPPKPKDTLMISRTPEVTCVVVDVSHEDPEVQFNWYVDGVEVHNAKTKPREEQFNSTFRVVSVLTVVHQDWLNGKEYKCKVSNKGLPAPIEKTISKTKGQPREPQVYTLPPSREEMTKNQVSLTCLVKGFYPSDIAVEWESNGQPENNYKTTPPMLDSDGSFFLYSKLTVDKSRWQQGNVFSCSVMHEALHNHYTQKSLSLSPGK

SEQ ID NO: 43 - protein, 516 aa, Artificial Sequence
  Description of Artificial Sequence: Synthetic polypeptide
CWLRQAKNGRCQVLYKTELSKEECCSTGRLSTSWTEEDVNDNTLFKWMIFNGGAPNCIPCKETCENVDCGPGKKCRMNKKNKPRCVCAPDCSNITWKGPVCGLDGKTYRNECALLKARCKEQPELEVQYQGRCKKTCRDVFCPGSSTCVVDQTNNAYCVTCNRICPEPASSEQYLCGNDGVTYSSACHLRKATCLLGRSIGLAYEGKCIKAKSCEDIQCTGGKKCLWDFKVGRGRCSLCDELCPDSKSDEPVCASDNATYASECAMKEAACSSGVLLEVKHSGSCNSISTGGGVECPPCPAPPVAGPSVFLFPPKPKDTLMISRTPEVTCVVVDVSHEDPEVQFNWYVDGVEVHNAKTKPREEQFNSTFRVVSVLTVVHQDWLNGKEYKCKVSNKGLPAPIEKTISKTKGQPREPQVYTLPPSREEMTKNQVSLTCLVKGFYPSDIAVEWESNGQPENNYKTTPPMLDSDGSFFLYSKLTVDKSRWQQGNVFSCSVMHEALHNHYTQKSLSLSPGK

SEQ ID NO: 44 - DNA, 1641 bp, Artificial Sequence
  Description of Artificial Sequence: Synthetic polynucleotide
atggtccgcgcgaggcaccagccgggtgggctttgcctcctgctgctgctgctctgccagttcatggaggaccgcagtgcccaggctgggaactgctggctccgtcaagcgaagaacggccgctgccaggtcctgtacaagaccgaactgagcaaggaggagtgctgcagcaccggccggctgagcacctcgtggaccgaggaggacgtgaatgacaacacactcttcaagtggatgattttcaacgggggcgcccccaactgcatcccctgtaaagaaacgtgtgagaacgtggactgtggacctgggaaaaaatgccgaatgaacaagaagaacaaaccccgctgcgtctgcgccccggattgttccaacatcacctggaagggtccagtctgcgggctggatgggaaaacctaccgcaatgaatgtgcactcctaaaggcaagatgtaaagagcagccagaactggaagtccagtaccaaggcagatgtaaaaagacttgtcgggatgttttctgtccaggcagctccacatgtgtggtggaccagaccaataatgcctactgtgtgacctgtaatcggatttgcccagagcctgcttcctctgagcaatatctctgtgggaatgatggagtcacctactccagtgcctgccacctgagaaaggctacctgcctgctgggcagatctattggattagcctatgagggaaagtgtatcaaagcaaagtcctgtgaagatatccagtgcactggtgggaaaaaatgtttatgggatttcaaggttgggagaggccggtgttccctctgtgatgagctgtgccctgacagtaagtcggatgagcctgtctgtgccagtgacaatgccacttatgccagcgagtgtgccatgaaggaagctgcctgctcctcaggtgtgctactggaagtaaagcactccggatcttgcaacaccggtggtggagtcgagtgcccaccgtgcccagcaccacctgtggcaggaccgtcagtcttcctcttccccccaaaacccaaggacaccctcatgatctcccggacccctgaggtcacgtgcgtggtggtggacgtgagccacgaagaccccgaggtccagttcaactggtacgtggacggcgtggaggtgcataatgccaagacaaagccacgggaggagcagttcaacagcacgttccgtgtggtcagcgtcctcaccgtcgtgcaccaggactggctgaacggcaaggagtacaagtgcaaggtctccaacaaaggcctcccagcccccatcgagaaaaccatctccaaaaccaaagggcagccccgagaaccacaggtgtacaccctgcccccatcccgggaggagatgaccaagaaccaggtcagcctgacctgcctggtcaaaggcttctaccccagcgacatcgccgtggagtgggagagcaatgggcagccggagaacaactacaagaccacacctcccatgctggactccgacggctccttcttcctctacagcaagctcaccgtggacaagagcaggtggcagcaggggaacgtcttctcatgctccgtgatgcatgaggctctgcacaaccactacacgcagaagagcctctccctgtctccgggtaaatgagaattc

SEQ ID NO: 45 - DNA, 1722 bp, Artificial Sequence
  Description of Artificial Sequence: Synthetic polynucleotide
atggtccgcgcgaggcaccagccgggtgggctttgcctcctgctgctgctgctctgccagttcatggaggaccgcagtgcccaggctgggaactgctggctccgtcaagcgaagaacggccgctgccaggtcctgtacaagaccgaactgagcaaggaggagtgctgcagcaccggccggctgagcacctcgtggaccgaggaggacgtgaatgacaacacactcttcaagtggatgattttcaacgggggtgcccccaactgcatcccctgtaaagaaacgtgtgagaacgtggactgtggacctgggaaaaaatgccgaatgaacaagaagaacaaaccccgctgcgtctgcgccccggattgttccaacatcacctggaagggtccagtctgcgggctggatgggaaaacctaccgcaatgaatgtgcactcctaaaggcaagatgtaaagagcagccagaactggaagtccagtaccaaggcagatgtaaaaagacttgtcgggatgttttctgtccaggcagctccacatgtgtggtggaccagaccaataatgcctactgtgtgacctgtaatcggatttgcccagagcctgcttcctctgagcaatatctctgtgggaatgatggagtcacctactccagtgcctgccacctgagaaaggctacctgcctgctgggcagatctattggattagcctatgagggaaagtgtatcaaagcaaagtcctgtgaagatatccagtgcactggtgggaaaaaatgtttatgggatttcaaggttgggagaggccggtgttccctctgtgatgagctgtgccctgacagtaagtcggatgagcctgtctgtgccagtgacaatgccacttatgccagcgagtgtgccatgaaggaagctgcctgctcctcaggtgtgctactggaagtaaagcactccggatcttgcaactccatttcggaagacaccgaggaagaggaggaagatgaagaccaggactacagctttcctatatcttctattctagagtggaccggtggtggagtcgagtgcccaccgtgcccagcaccacctgtggcaggaccgtcagtcttcctcttccccccaaaacccaaggacaccctcatgatctcccggacccctgaggtcacgtgcgtggtggtggacgtgagccacgaagaccccgaggtccagttcaactggtacgtggacggcgtggaggtgcataatgccaagacaaagccacgggaggagcagttcaacagcacgttccgtgtggtcagcgtcctcaccgtcgtgcaccaggactggctgaacggcaaggagtacaagtgcaaggtctccaacaaaggcctcccagcccccatcgagaaaaccatctccaaaaccaaagggcagccccgagaaccacaggtgtacaccctgcccccatcccgggaggagatgaccaagaaccaggtcagcctgacctgcctggtcaaaggcttctaccccagcgacatcgccgtggagtgggagagcaatgggcagccggagaacaactacaagaccacacctcccatgctggactccgacggctccttcttcctctacagcaagctcaccgtggacaagagcaggtggcagcaggggaacgtcttctcatgctccgtgatgcatgaggctctgcacaaccactacacgcagaagagcctctccctgtctccgggtaaatgagaattc

SEQ ID NO: 46 - protein, 4 aa, Artificial Sequence
  Description of Artificial Sequence: Synthetic peptide
TGGG

SEQ ID NO: 47 - protein, 6 aa, Artificial Sequence
  Description of Artificial Sequence: Synthetic 6xHis tag
HHHHHH